European Patent Specification EP 3 421 493 B1, published January 17, 2024. Title: MONOCLONAL ANTIBODIES TO PROGASTRIN AND THEIR USES. Applicant: Progastrine et Cancers S.à r.l. CENTRE NATIONAL DE LA RECHERCHE SCIENTIFIQUE (CNRS) INSTITUT NATIONAL DE LA SANTE ET DE LA RECHERCHE MEDICALE (INSERM). Application PCT/EP2010/006329. The sequence listing filed with the application follows.

SEQUENCE LISTING (99 sequences)

SEQ ID NO: 1 - protein, 8 aa, Artificial Sequence
  source: /note="Description of Artificial Sequence: Synthetic peptide"
GYIFTSYW

SEQ ID NO: 2 - protein, 8 aa, Artificial Sequence
  source: /note="Description of Artificial Sequence: Synthetic peptide"
FYPGNSDS

SEQ ID NO: 3 - protein, 8 aa, Artificial Sequence
  source: /note="Description of Artificial Sequence: Synthetic peptide"
TRRDSPQY

SEQ ID NO: 4 - protein, 11 aa, Artificial Sequence
  source: /note="Description of Artificial Sequence: Synthetic peptide"
QSIVHSNGNTY

SEQ ID NO: 5 - protein, 3 aa, Artificial Sequence
  source: /note="Description of Artificial Sequence: Synthetic peptide"
KVS

SEQ ID NO: 6 - protein, 9 aa, Artificial Sequence
  source: /note="Description of Artificial Sequence: Synthetic peptide"
FQGSHVPFT

SEQ ID NO: 7 - protein, 8 aa, Artificial Sequence
  source: /note="Description of Artificial Sequence: Synthetic peptide"
GYTFSSSW

SEQ ID NO: 8 - protein, 8 aa, Artificial Sequence
  source: /note="Description of Artificial Sequence: Synthetic peptide"
FLPGSGST

SEQ ID NO: 9 - protein, 11 aa, Artificial Sequence
  source: /note="Description of Artificial Sequence: Synthetic peptide"
ATDGNYDWFAY

SEQ ID NO: 10 - protein, 11 aa, Artificial Sequence
  source: /note="Description of Artificial Sequence: Synthetic peptide"
QSLVHSSGVTY

SEQ ID NO: 11 - protein, 9 aa, Artificial Sequence
  source: /note="Description of Artificial Sequence: Synthetic peptide"
SQSTHVPPT

SEQ ID NO: 12 - protein, 115 aa, Artificial Sequence
  source: /note="Description of Artificial Sequence: Synthetic polypeptide"
EVQLQQSGTVLARPGASVKMSCKASGYIFTSYWVHWVKQRPGQGLEWIGGFYPGNSDSRYNQKFKGKATLTAVTSASTAYMDLSSLTNEDSAVYFCTRRDSPQYWGQGTTLTVSS

SEQ ID NO: 13 - protein, 112 aa, Artificial Sequence
  source: /note="Description of Artificial Sequence: Synthetic polypeptide"
DVLMTQTPLSLPVSLGDQASISCRSSQSIVHSNGNTYLEWYLQKPGQSPKLLIYKVSNRFSGVPDRFSGSGSGTDFTLKISRLEAEDLGVYYCFQGSHVPFTFGGGTKLEIK

SEQ ID NO: 14 - protein, 118 aa, Artificial Sequence
  source: /note="Description of Artificial Sequence: Synthetic polypeptide"
QVQLQQSGAELMKPGASVKISCKATGYTFSSSWIEWLKQRPGHGLEWIGEFLPGSGSTDYNEKFKGKATFTADTSSDTAYMLLSSLTSEDSAVYYCATDGNYDWFAYWGQGTLVTVSA

SEQ ID NO: 15 - protein, 112 aa, Artificial Sequence
  source: /note="Description of Artificial Sequence: Synthetic polypeptide"
DLVMTQTPLSLPVSLGDQASISCRSSQSLVHSSGVTYLHWYLQKPGQSPKLLIYKVSNRFSGVPDRFSGSGSGTDFTLKISRVEAEDLGVYFCSQSTHVPPTFGSGTKLEIK

SEQ ID NO: 16 - DNA, 345 bp, Artificial Sequence
  source: /note="Description of Artificial Sequence: Synthetic polynucleotide"
  CDS (1)..(345)
gaggttcagctccagcagtctgggactgtgctggcaaggcctggggcttccgtgaagatgtcctgcaaggcttctggctacatctttaccagctactgggtacactgggttaaacagaggcctggacagggtctagaatggattggtggtttttatcctggaaatagtgattctaggtacaaccagaaattcaagggcaaggccacactgactgcagtcacatccgccagtactgcctacatggacctcagcagcctgacaaatgaggactctgcggtctatttctgtacaagaagagatagtccccagtactggggccaaggcaccactctcacagtctcctca

SEQ ID NO: 17 - DNA, 336 bp, Artificial Sequence
  source: /note="Description of Artificial Sequence: Synthetic polynucleotide"
  CDS (1)..(336)
gatgttttgatgacccaaactccactctccctgcctgtcagtcttggagatcaagcctccatctcttgcagatctagtcagagcattgtacatagtaatggaaacacctatttagaatggtacctgcagaaaccaggccagtctccaaagctcctgatctacaaagtttccaaccgattttctggggtcccagacaggttcagtggcagtggatcagggacagatttcacactcaagatcagcagactggaggctgaggatctgggagtttattactgctttcaaggttcacatgttccgttcacgttcggaggggggaccaagctggaaataaaa

SEQ ID NO: 18 - DNA, 354 bp, Artificial Sequence
  source: /note="Description of Artificial Sequence: Synthetic polynucleotide"
  CDS (1)..(354)
caggttcagttgcagcagtctggagctgagctgatgaagccaggggcctcagtgaagatatcctgcaaggctactggctacacattcagtagctcctggatagagtggttaaaacagaggcctggacatggccttgagtggattggagagtttttacctggaagtggtagtacagactacaatgagaagttcaagggcaaggccacattcactgcagacacatcctccgacacagcctacatgctactcagcagcctgacatctgaggactctgccgtctattactgtgcaactgatggtaattatgactggtttgcttactggggccaagggactctggtcactgtctctgca

SEQ ID NO: 19 - DNA, 336 bp, Artificial Sequence
  source: /note="Description of Artificial Sequence: Synthetic polynucleotide"
  CDS (1)..(336)
gatcttgtgatgacccaaactccactctccctgcctgtcagtcttggagatcaagcctccatctcttgcagatctagtcagagccttgtacacagtagtggagtcacctatttacattggtacctgcagaagccaggccagtctccaaagctcctgatctacaaagtttccaaccgattttctggggtcccagacaggttcagtggcagtggatcagggacagatttcacactcaagatcagcagagtggaggctgaggatctgggagtttatttctgctctcaaagtacacatgttcctcccacgttcggctcggggacaaagttggaaataaaa

SEQ ID NO: 20 - protein, 80 aa, Homo sapiens
SWKPRSQQPDAPLGTGANRDLELPWLEQQGPASHHRRQLGPQGPPHLVADPSKKQGPWLEEEEEAYGWMDFGRRSAEDEN

SEQ ID NO: 21 - protein, 115 aa, Artificial Sequence
  source: /note="Description of Artificial Sequence: Synthetic polypeptide"
QVQLVQSGAEVKKPGASVKVSCKASGYIFTSYWVHWVRQAPGQRLEWMGGFYPGNSDSRYSQKFQGRVTITRDTSASTAYMELSSLRSEDTAVYYCTRRDSPQYWGQGTLVTVSS

SEQ ID NO: 22 - protein, 112 aa, Artificial Sequence
  source: /note="Description of Artificial Sequence: Synthetic polypeptide"
DVVMTQSPLSLPVTLGQPASISCRSSQSIVHSNGNTYLEWFQQRPGQSPRRLIYKVSNRFSGVPDRFSGSGSGTDFTLKISRVEAEDVGVYYCFQGSHVPFTFGGGTKVEIK

SEQ ID NO: 23 - protein, 118 aa, Artificial Sequence
  source: /note="Description of Artificial Sequence: Synthetic polypeptide"
QVQLVQSGAEVKKPGASVKVSCKASGYTFSSSWMHWVRQAPGQGLEWMGIFLPGSGSTDYAQKFQGRVTMTRDTSTSTVYMELSSLRSEDTAVYYCATDGNYDWFAYWGQGTLVTVSS

SEQ ID NO: 24 - protein, 112 aa, Artificial Sequence
  source: /note="Description of Artificial Sequence: Synthetic polypeptide"
DIVMTQTPLSLSVTPGQPASISCKSSQSLVHSSGVTYLYWYLQKPGQSPQLLIYKVSNRFSGVPDRFSGSGSGTDFTLKISRVEAEDVGVYYCSQSTHVPPTFGQGTKLEIK

SEQ ID NO: 25 - protein, 14 aa, Homo sapiens
SWKPRSQQPDAPLG

SEQ ID NO: 26 - protein, 16 aa, Artificial Sequence
  source: /note="Description of Artificial Sequence: Synthetic peptide"
  MOD_RES (15)..(15): Ahx
SWKPRSQQPDAPLGXC

SEQ ID NO: 27 - protein, 26 aa, Homo sapiens
QGPWLEEEEEAYGWMDFGRRSAEDEN

SEQ ID NO: 28 - protein, 5 aa, Homo sapiens
DAPLG

SEQ ID NO: 29 - protein, 6 aa, Homo sapiens
PDAPLG

SEQ ID NO: 30 - protein, 7 aa, Homo sapiens
PRSQQPD

SEQ ID NO: 31 - protein, 9 aa, Homo sapiens
WKPRSQQPD

SEQ ID NO: 32 - protein, 13 aa, Homo sapiens
WKPRSQQPDAPLG

SEQ ID NO: 33 - protein, 4 aa, Homo sapiens
FGRR

SEQ ID NO: 34 - protein, 5 aa, Homo sapiens
MDFGR

SEQ ID NO: 35 - protein, 5 aa, Homo sapiens
AEDEN

SEQ ID NO: 36 - protein, 8 aa, Homo sapiens
GWMDFGRR

SEQ ID NO: 37 - protein, 8 aa, Artificial Sequence
  source: /note="Description of Artificial Sequence: Synthetic peptide"
GFTFTTYA

SEQ ID NO: 38 - protein, 8 aa, Artificial Sequence
  source: /note="Description of Artificial Sequence: Synthetic peptide"
GFIFSSYG

SEQ ID NO: 39 - protein, 8 aa, Artificial Sequence
  source: /note="Description of Artificial Sequence: Synthetic peptide"
GYTFTSYY

SEQ ID NO: 40 - protein, 9 aa, Artificial Sequence
  source: /note="Description of Artificial Sequence: Synthetic peptide"
GYSITSDYA

SEQ ID NO: 41 - protein, 8 aa, Artificial Sequence
  source: /note="Description of Artificial Sequence: Synthetic peptide"
ISSGGTYT

SEQ ID NO: 42 - protein, 8 aa, Artificial Sequence
  source: /note="Description of Artificial Sequence: Synthetic peptide"
INTFGDRT

SEQ ID NO: 43 - protein, 8 aa, Artificial Sequence
  source: /note="Description of Artificial Sequence: Synthetic peptide"
INPSNGGT

SEQ ID NO: 44 - protein, 7 aa, Artificial Sequence
  source: /note="Description of Artificial Sequence: Synthetic peptide"
ISFSGYT

SEQ ID NO: 45 - protein, 10 aa, Artificial Sequence
  source: /note="Description of Artificial Sequence: Synthetic peptide"
ATQGNYSLDF

SEQ ID NO: 46 - protein, 7 aa, Artificial Sequence
  source: /note="Description of Artificial Sequence: Synthetic peptide"
ARGTGTY

SEQ ID NO: 47 - protein, 10 aa, Artificial Sequence
  source: /note="Description of Artificial Sequence: Synthetic peptide"
TRGGYYPFDY

SEQ ID NO: 48 - protein, 14 aa, Artificial Sequence
  source: /note="Description of Artificial Sequence: Synthetic peptide"
AREVNYGDSYHFDY

SEQ ID NO: 49 - protein, 11 aa, Artificial Sequence
  source: /note="Description of Artificial Sequence: Synthetic peptide"
KSLRHTKGITF

SEQ ID NO: 50 - protein, 11 aa, Artificial Sequence
  source: /note="Description of Artificial Sequence: Synthetic peptide"
QSLLDSDGKTY

SEQ ID NO: 51 - protein, 7 aa, Artificial Sequence
  source: /note="Description of Artificial Sequence: Synthetic peptide"
SQHRTYT

SEQ ID NO: 52 - protein, 3 aa, Artificial Sequence
  source: /note="Description of Artificial Sequence: Synthetic peptide"
QMS

SEQ ID NO: 53 - protein, 3 aa, Artificial Sequence
  source: /note="Description of Artificial Sequence: Synthetic peptide"
LVS

SEQ ID NO: 54 - protein, 7 aa, Artificial Sequence
  source: /note="Description of Artificial Sequence: Synthetic peptide"
VKKDGSH

SEQ ID NO: 55 - protein, 9 aa, Artificial Sequence
  source: /note="Description of Artificial Sequence: Synthetic peptide"
AQNLELPLT

SEQ ID NO: 56 - protein, 9 aa, Artificial Sequence
  source: /note="Description of Artificial Sequence: Synthetic peptide"
WQGTHFPQT

SEQ ID NO: 57 - protein, 9 aa, Artificial Sequence
  source: /note="Description of Artificial Sequence: Synthetic peptide"
WQGTHSPYT

SEQ ID NO: 58 - protein, 13 aa, Artificial Sequence
  source: /note="Description of Artificial Sequence: Synthetic peptide"
GVGDAIKGQSVFV

SEQ ID NO: 59 - protein, 117 aa, Artificial Sequence
  source: /note="Description of Artificial Sequence: Synthetic polypeptide"
EVQLVESGGGLVKPGGSLKLSCAASGFTFTTYAMSWVRQTPEKRLEWVATISSGGTYTYYPDSVKGRFTISRDNAKNALYLQMSSLRSEDTAMYYCATQGNYSLDFWGQGTSLTVSS

SEQ ID NO: 60 - protein, 114 aa, Artificial Sequence
  source: /note="Description of Artificial Sequence: Synthetic polypeptide"
EVQLVESGGGLVQPGGSLKLSCAASGFIFSSYGMSWVRQSPDRRLELVASINTFGDRTYYPDSVKGRFTISRDNAKNTLYLQMTSLKSEDTAIYYCARGTGTYWGQGTTLTVSS

SEQ ID NO: 61 - protein, 117 aa, Artificial Sequence
  source: /note="Description of Artificial Sequence: Synthetic polypeptide"
QVQLQQSGAELVKPGASVKLSCKASGYTFTSYYMYWVKQRPGQGLEWIGEINPSNGGTNFNEKFKSKATLTVDKSSSTAYMQLSSLTSEDSAVYYCTRGGYYPFDYWGQGTTLTVSS

SEQ ID NO: 62 - protein, 121 aa, Artificial Sequence
  source: /note="Description of Artificial Sequence: Synthetic polypeptide"
DVQLQESGPGLVKPSQSLSLTCTVTGYSITSDYAWNWIRQFPGNKLEWMGYISFSGYTSYNPSLKSRISVTRDTSRNQFFLQLTSVTTEDTATYYCAREVNYGDSYHFDYWGQGTIVTVSS

SEQ ID NO: 63 - protein, 112 aa, Artificial Sequence
  source: /note="Description of Artificial Sequence: Synthetic polypeptide"
DIVMTQAASSNPVTLGTSASISCRSSKSLRHTKGITFLYWYLQKPGQSPQLLIYQMSNLASGVPDRFSSSGSGTDFTLRISRVEAEDLGVYYCAQNLELPLTFGAGTKLELK

SEQ ID NO: 64 - protein, 112 aa, Artificial Sequence
  source: /note="Description of Artificial Sequence: Synthetic polypeptide"
DVVLTQTPLTLSVTIGQPASISCKSSQSLLDSDGKTYLNWLLQRPGQSPKRLIYLVSKLDSGVPDRFTGSGSGTDFTLKISRVEAEDLGVYYCWQGTHFPQTFGGGTKLEIK

SEQ ID NO: 65 - protein, 112 aa, Artificial Sequence
  source: /note="Description of Artificial Sequence: Synthetic polypeptide"
DVVMTQTPLTLSVTIGRPASISCKSSQSLLDSDGKTYLYWLLQRPGQSPKRLIYLVSELDSGVPDRITGSGSGTDFTLKISRVEAEDLGVYYCWQGTHSPYTFGGGTKLEIK

SEQ ID NO: 66 - protein, 115 aa, Artificial Sequence
  source: /note="Description of Artificial Sequence: Synthetic polypeptide"
QLALTQSSSASFSLGASAKLTCTLSSQHRTYTIEWYQQQSLKPPKYVMEVKKDGSHSTGHGIPDRFSGSSSGADRYLSISNIQPEDEAIYICGVGDAIKGQSVFVFGGGTKVTVL

SEQ ID NO: 67 - DNA, 351 bp, Artificial Sequence
  source: /note="Description of Artificial Sequence: Synthetic polynucleotide"
  CDS (1)..(351)
gaagtgcagctggtggagtctgggggaggcttagtgaagcctggagggtccctgaaactctcctgtgcagcctctggattcactttcactacctatgccatgtcttgggttcgccagactccggagaagaggctggagtgggtcgcaaccattagtagtggtggtacttacacctactatccagacagtgtgaagggtcgattcaccatctccagagacaatgccaagaacgccctatacctgcaaatgagcagtctgaggtctgaggacacggccatgtattactgtgcaacacaggggaattactctttggacttctggggccaaggcacctctctcacagtctcctca

SEQ ID NO: 68 - DNA, 342 bp, Artificial Sequence
  source: /note="Description of Artificial Sequence: Synthetic polynucleotide"
  CDS (1)..(342)
gaggtgcagctggtggagtctgggggaggcttggtgcagcctggagggtccctgaaactctcctgtgcagcctctggattcattttcagtagctatggcatgtcttgggttcgccagtctccagacaggaggctggagttggtcgcaagtattaatacttttggtgatagaacctattatccagacagtgtgaagggccgattcaccatctccagagacaatgccaagaacaccctgtacctgcaaatgaccagtctgaagtctgaggacacagccatttattactgtgcaagagggaccggaacctactggggccaaggcaccactctcacagtctcctca

SEQ ID NO: 69 - DNA, 351 bp, Artificial Sequence
  source: /note="Description of Artificial Sequence: Synthetic polynucleotide"
  CDS (1)..(351)
caggtccaactgcagcagtctggggctgaactggtgaagcctggggcttcagtgaagttgtcctgcaaggcttctggctacaccttcaccagctactatatgtactgggtgaagcagaggcctggacaaggccttgagtggattggagagattaatcctagcaatggtggtactaacttcaatgagaagttcaagagcaaggccacactgactgtagacaaatcctccagcacagcatacatgcaactcagcagcctgacatctgaggactctgcggtctattactgtacaagaggcggttactacccctttgactactggggccaaggcaccactctcacagtctcctca

SEQ ID NO: 70 - DNA, 363 bp, Artificial Sequence
  source: /note="Description of Artificial Sequence: Synthetic polynucleotide"
  CDS (1)..(363)
gatgtgcagcttcaggagtcgggacctggcctggtgaaaccttctcagtctctgtccctcacatgcactgtcactggctactcaatcaccagtgattatgcctggaattggatccggcagtttccaggaaacaaactggagtggatgggctacataagcttcagtggttacactagttacaacccatctctcaaaagtcgaatctctgtcactcgggacacatccaggaaccaattcttcctccagttgacttctgtgactactgaggacacagccacatattactgtgcaagagaggtcaactatggggactcctaccactttgactactggggccaaggcaccattgtcacagtctcctca

SEQ ID NO: 71 - DNA, 336 bp, Artificial Sequence
  source: /note="Description of Artificial Sequence: Synthetic polynucleotide"
  CDS (1)..(336)
gacattgtgatgacgcaggctgcatcctctaatccagtcactcttggaacatccgcttccatctcctgcaggtctagtaagagtctccgacatactaaaggcatcacttttttgtattggtatctgcagaagccaggccagtctcctcagctcctgatttatcagatgtccaaccttgcctcaggagtcccagacaggttcagtagcagtgggtcaggaactgatttcacactgagaatcagcagagtggaggctgaggatttgggtgtttattactgtgctcaaaatctagaacttccgctcacgttcggtgctgggaccaagctggagctgaaa

SEQ ID NO: 72 - DNA, 336 bp, Artificial Sequence
  source: /note="Description of Artificial Sequence: Synthetic polynucleotide"
  CDS (1)..(336)
gatgttgtgctgacccagactccactcactttgtcggttaccattggacaaccagcctccatctcctgcaagtcaagtcagagcctcttagatagtgatggaaagacatatttgaattggttgttacagaggccaggccagtctccaaagcgcctaatctatctggtgtctaaactggactctggagtccctgacaggttcactggcagtggatcagggacagatttcacactgaaaatcagcagagtggaggctgaggatttgggagtttattattgctggcaaggtacacattttcctcagacgttcggtggaggcaccaagctggaaatcaaa

SEQ ID NO: 73 - DNA, 336 bp, Artificial Sequence
  source: /note="Description of Artificial Sequence: Synthetic polynucleotide"
  CDS (1)..(336)
gatgttgtgatgacccagactccactcactttgtcggttaccattgggcgcccagcctccatctcttgcaagtcaagtcagagcctcttagacagtgatggaaagacatatttgtattggttgttacagaggccaggccagtctccaaagcgcctaatctatctggtgtctgagctggactctggagtccctgacaggatcactggcagtgggtcggggacagatttcacactgaagatcagcagagtggaggctgaggatttgggagtttattattgctggcaaggaacacattctccgtacacgttcggaggggggaccaagctggaaataaaa

SEQ ID NO: 74 - DNA, 345 bp, Artificial Sequence
  source: /note="Description of Artificial Sequence: Synthetic polynucleotide"
  CDS (1)..(345)
caacttgcgctcactcagtcatcttcagcctctttctccctgggagcctcagcaaaactaacgtgcactttgagtagtcaacacagaacgtacaccattgaatggtatcagcaacagtcactcaagcctcctaagtatgtgatggaggttaagaaagatggaagccacagcacaggtcatgggattcctgatcgcttctctggatccagttctggtgctgatcgctacctcagcatttccaacatccagcctgaagatgaagcaatatacatctgtggtgtgggtgatgcaattaagggacaatctgtgtttgttttcggcggtggcaccaaggtcactgtccta

SEQ ID NO: 75 - protein, 117 aa, Artificial Sequence
  source: /note="Description of Artificial Sequence: Synthetic polypeptide"
EVQLVESGGGLVKPGGSLRLSCAASGFTFTTYAMSWVRQAPGKGLEWVSSISSGGTYTYYADSVKGRFTISRDNAKNSLYLQMNSLRAEDTAVYYCATQGNYSLDFWGQGTTVTVSS

SEQ ID NO: 76 - protein, 112 aa, Artificial Sequence
  source: /note="Description of Artificial Sequence: Synthetic polypeptide"
DIVMTQSPLSLPVTPGEPASISCRSSKSLRHTKGITFLYWYLQKPGQSPQLLIYQMSNRASGVPDRFSGSGSGTDFTLKISRVEAEDVGVYYCAQNLELPLTFGGGTKVEIK

SEQ ID NO: 77 - protein, 117 aa, Artificial Sequence
  source: /note="Description of Artificial Sequence: Synthetic polypeptide"
EVQLVESGGGLVKPGGSLRLSCAASGFTFTTYAMNWVRQAPGKGLEWVSSISSGGTYTYYADSVKGRFTISRDNAKNSLYLQMNSLRAEDTAVYYCATQGNYSLDFWGQGTTVTVSS

SEQ ID NO: 78 - protein, 112 aa, Artificial Sequence
  source: /note="Description of Artificial Sequence: Synthetic polypeptide"
DIVMTQSPLSLPVTPGEPASISCRSSKSLRHTKGITFLDWYLQKPGQSPQLLIYQMSNRASGVPDRFSGSGSGTDFTLKISRVEAEDVGVYYCAQNLELPLTFGGGTKVEIK

SEQ ID NO: 79 - protein, 117 aa, Artificial Sequence
  source: /note="Description of Artificial Sequence: Synthetic polypeptide"
EVQLVESGGGLVKPGGSLRLSCAASGFTFTTYAMSWVRQAPGKGLEWVSTISSGGTYTYYADSVKGRFTISRDNAKNSLYLQMNSLRAEDTAVYYCATQGNYSLDFWGQGTTVTVSS

SEQ ID NO: 80 - protein, 114 aa, Artificial Sequence
  source: /note="Description of Artificial Sequence: Synthetic polypeptide"
EVQLVESGGGLVQPGGSLRLSCAASGFIFSSYGMSWVRQAPGKGLEWVANINTFGDRTYYVDSVKGRFTISRDNAKNSLYLQMNSLRAEDTAVYYCARGTGTYWGQGTLVTVSS

SEQ ID NO: 81 - protein, 112 aa, Artificial Sequence
  source: /note="Description of Artificial Sequence: Synthetic polypeptide"
DVVMTQSPLSLPVTLGQPASISCRSSQSLLDSDGKTYLNWFQQRPGQSPRRLIYLVSNRDSGVPDRFSGSGSGTDFTLKISRVEAEDVGVYYCWQGTHFPQTFGGGTKVEIK

SEQ ID NO: 82 - protein, 114 aa, Artificial Sequence
  source: /note="Description of Artificial Sequence: Synthetic polypeptide"
EVQLVESGGGLVQPGGSLRLSCAASGFIFSSYGMSWVRQAPGKGLEWVASINTFGDRTYYVDSVKGRFTISRDNAKNSLYLQMNSLRAEDTAVYYCARGTGTYWGQGTLVTVSS

SEQ ID NO: 83 - protein, 112 aa, Artificial Sequence
  source: /note="Description of Artificial Sequence: Synthetic polypeptide"
DVVMTQSPLSLPVTLGQPASISCRSSQSLLDSDGKTYLNWFQQRPGQSPRRLIYLVSKRDSGVPDRFSGSGSGTDFTLKISRVEAEDVGVYYCWQGTHFPQTFGGGTKVEIK

SEQ ID NO: 84 - protein, 117 aa, Artificial Sequence
  source: /note="Description of Artificial Sequence: Synthetic polypeptide"
QVQLVQSGAEVKKPGASVKVSCKASGYTFTSYYMYWVRQAPGQGLEWMGIINPSNGGTSYAQKFQGRVTMTRDTSTSTVYMELSSLRSEDTAVYYCTRGGYYPFDYWGQGTTVTVSS

SEQ ID NO: 85 - protein, 112 aa, Artificial Sequence
  source: /note="Description of Artificial Sequence: Synthetic polypeptide"
DVVMTQSPLSLPVTLGQPASISCRSSQSLLDSDGKTYLYWFQQRPGQSPRRLIYLVSNRDSGVPDRFSGSGSGTDFTLKISRVEAEDVGVYYCWQGTHSPYTFGQGTKLEIK

SEQ ID NO: 86 - protein, 117 aa, Artificial Sequence
  source: /note="Description of Artificial Sequence: Synthetic polypeptide"
QVQLVQSGAEVKKPGASVKVSCKASGYTFTSYYMHWVRQAPGQGLEWMGIINPSNGGTSYAQKFQGRVTMTRDTSTSTVYMELSSLRSEDTAVYYCTRGGYYPFDYWGQGTTVTVSS

SEQ ID NO: 87 - protein, 112 aa, Artificial Sequence
  source: /note="Description of Artificial Sequence: Synthetic polypeptide"
DVVMTQSPLSLPVTLGQPASISCRSSQSLLDSDGKTYLNWFQQRPGQSPRRLIYLVSNRDSGVPDRFSGSGSGTDFTLKISRVEAEDVGVYYCWQGTHSPYTFGQGTKLEIK

SEQ ID NO: 88 - protein, 117 aa, Artificial Sequence
  source: /note="Description of Artificial Sequence: Synthetic polypeptide"
QVQLVQSGAEVKKPGASVKVSCKASGYTFTSYYMYWVRQAPGQGLEWMGEINPSNGGTNYAQKFQGRVTMTRDTSTSTVYMELSSLRSEDTAVYYCTRGGYYPFDYWGQGTTVTVSS

SEQ ID NO: 89 - protein, 112 aa, Artificial Sequence
  source: /note="Description of Artificial Sequence: Synthetic polypeptide"
DVVMTQSPLSLPVTLGQPASISCRSSQSLLDSDGKTYLYWFQQRPGQSPRRLIYLVSERDSGVPDRFSGSGSGTDFTLKISRVEAEDVGVYYCWQGTHSPYTFGQGTKLEIK

SEQ ID NO: 90 - protein, 121 aa, Artificial Sequence
  source: /note="Description of Artificial Sequence: Synthetic polypeptide"
QVQLQESGPGLVKPSQTLSLTCTVSGYSITSDYAWNWIRQHPGKGLEWIGYISFSGYTYYNPSLKSRVTISVDTSKNQFSLKLSSVTAADTAVYYCAREVNYGDSYHFDYWGQGTLVTVSS

SEQ ID NO: 91 - protein, 115 aa, Artificial Sequence
  source: /note="Description of Artificial Sequence: Synthetic polypeptide"
QLVLTQSPSASASLGASVKLTCTLSSQHRTYTIEWHQQQPEKGPRYLMKVKKDGSHSKGDGIPDRFSGSSSGAERYLTISSLQSEDEADYYCGVGDAIKGQSVFVFGGGTKVEIK

SEQ ID NO: 92 - protein, 121 aa, Artificial Sequence
  source: /note="Description of Artificial Sequence: Synthetic polypeptide"
QVQLQESGPGLVKPSQTLSLTCTVSGYSITSDYAWSWIRQHPGKGLEWIGYISFSGYTYYNPSLKSRVTISVDTSKNQFSLKLSSVTAADTAVYYCAREVNYGDSYHFDYWGQGTLVTVSS

SEQ ID NO: 93 - protein, 115 aa, Artificial Sequence
  source: /note="Description of Artificial Sequence: Synthetic polypeptide"
QLVLTQSPSASASLGASVKLTCTLSSQHRTYTIAWHQQQPEKGPRYLMKVKKDGSHSKGDGIPDRFSGSSSGAERYLTISSLQSEDEADYYCGVGDAIKGQSVFVFGGGTKVEIK

SEQ ID NO: 94 - protein, 121 aa, Artificial Sequence
  source: /note="Description of Artificial Sequence: Synthetic polypeptide"
QVQLQESGPGLVKPSQTLSLTCTVSGYSITSDYAWNWIRQHPGKGLEWIGYISFSGYTSYNPSLKSRVTISVDTSKNQFSLKLSSVTAADTAVYYCAREVNYGDSYHFDYWGQGTLVTVSS

SEQ ID NO: 95 - protein, 115 aa, Artificial Sequence
  source: /note="Description of Artificial Sequence: Synthetic polypeptide"
QLVLTQSPSASASLGASVKLTCTLSSQHRTYTIEWHQQQPEKGPRYLMEVKKDGSHSKGDGIPDRFSGSSSGAERYLTISSLQSEDEADYYCGVGDAIKGQSVFVFGGGTKVEIK

SEQ ID NO: 96 - protein, 29 aa, Artificial Sequence
  source: /note="Description of Artificial Sequence: Synthetic peptide"
  MOD_RES (2)..(3): Ahx
CXXQGPWLEEEEEAYGWMDFGRRSAEDEN

SEQ ID NO: 97 - protein, 13 aa, Artificial Sequence
  source: /note="Description of Artificial Sequence: Synthetic peptide"
  MOD_RES (2)..(3): Ahx
CXXFGRRSAEDEN

SEQ ID NO: 98 - protein, 13 aa, Artificial Sequence
  source: /note="Description of Artificial Sequence: Synthetic peptide"
  MOD_RES (11)..(12): Ahx
FGRRSAEDENXXC

SEQ ID NO: 99 - protein, 15 aa, Artificial Sequence
  source: /note="Description of Artificial Sequence: Synthetic peptide"
GGGGSGGGGSGGGGS